European Patent Specification EP 3 845 642 B1, published August 9, 2023. Title: SERINE PROTEASES OF Bacillus Species. Applicant: Danisco US, Inc. Application DIVISIONAL APPLICATION OF: EP 17722562.0. The sequence listing filed with the application follows.

SEQUENCE LISTING (41 sequences)

SEQ ID NO: 1 - protein, 278 aa, artificial sequence
  truncated version of BspE04637 protease
AQTVPWGVPHVQGTDAHAAGHTGSGVKVAILDTGIDRNHEDLNVRGGHSVFTDSANRDPYYDGSGHGTHVAGTVAALNNSVGVLGVAYNAELYAVKVLNNSGSGSYAGIAEGIEWAVQNNMDIINMSLGGSMSSSILEEWCNIAYNSGVLVVAAAGNSGRTNGRGDTVGYPAKYDSVIAVAAVDSSNNRASFSSTGPAVEIAAPGVNILSTTPGNSYASYNGTSMASPHVAGVAALVLAANPNLSNVELRNRLNDTAQNLGDANHFGNGLVRAVDAIN

SEQ ID NO: 2 - DNA, 538 bp, Bacillus. subtilis
gaattctccattttcttctgctatcaaaataacagactcgtgattttccaaacgagctttcaaaaaagcctctgccccttgcaaatcggatgcctgtctataaaattcccgatattggttaaacagcggcgcaatggcggccgcatctgatgtctttgcttggcgaatgttcatcttatttcttcctccctctcaataattttttcattctatcccttttctgtaaagtttatttttcagaatacttttatcatcatgctttgaaaaaatatcacgataatatccattgttctcacggaagcacacgcaggtcatttgaacgaattttttcgacaggaatttgccgggactcaggagcatttaacctaaaaaagcatgacatttcagcataatgaacatttactcatgtctattttcgttcttttctgtatgaaaatagttatttcgagtctctacggaaatagcgagagatgatatacctaaatagagataaaatcatctcaaaaaaatgggtctactaaaatattattccatctat

SEQ ID NO: 3 - DNA, 87 bp, Bacillus. subtilis
gtgagaagcaaaaaattgtggatcagcttgttgtttgcgttaacgttaatctttacgatggcgttcagcaacatgtctgctagcgca

SEQ ID NO: 4 - protein, 29 aa, Bacillus. subtilis
VRSKKLWISLLFALTLIFTMAFSNMSAQA

SEQ ID NO: 5 - DNA, 216 bp, Bacillus sp.
  misc_feature (1)..(216): Bacillus sp. GX6638 (ATCC 53278)
caatcacaggctgaaaaacaggagtaccttgttcaatttaatgacaaggtaaataaggggatattaaacgcatttggtgtcgacaacagtgatgttcttcatacttacaatctactacctgttaatctagtaaaaatgacagagcagcaagcgaaagcattacaaaataatccgcatattaaagcggtggaacctaactttgaggcgcaagcattc

SEQ ID NO: 6 - protein, 72 aa, Bacillus sp.
  MISC_FEATURE (1)..(216): Bacillus sp. GX6638 (ATCC 53278)
QSQAEKQEYLVQFNDKVNKGILNAFGVDNSDVLHTYNLLPVNLVKMTEQQAKALQNNPHIKAVEPNFEAQAF

SEQ ID NO: 7 - DNA, 93 bp, Bacillus amyloliquefaciens
ggttaccttgaatgtatataaacattctcaaagggatttctaataaaaaacgctcggttgccgccgggcgttttttatgcatcgatggaattc

SEQ ID NO: 8 - DNA, 837 bp, artificial sequence
  BspE-clade protease variant
gctcaaacagtaccgtggggagttcctcatgttcaaggtactgatgctcatgcagcggggcatactggaagtggtgtaaaagtagctatactcgatacgggaattgatgctaatcatgaagatttaaatgtaagaggagggcactctgtattcacaggcagtgcaaacagagatccttattacgatggtagtggtcatggcacgcacgttgctggaacagtagcggccttaaataatagtgtaggtgtgttaggtgtagcctacaacgcggagctatatgcggtaaaagtattaaataaccgcggaagtggttcttatgcgggaatcgctgaaggaattgaatgggcagtacaaaaccgtatggacattataaatatgagtttaggaggttcgatgagttcttctattttagaagagtggtgtaatcgcgcctacaattctggtgtgcttgtagtggcggcagctggaaatagtggacgtacgaatggccgtgggaacactgttggttatccagcaaaatatgattctgttatcgcagtagcagcagtttcatctagcaacaatcgtgcaagtttctctagtacaggaaaggcagtggaaattgctgcaccaggtgtaaacattcttagtacgactcctggaaacagctatgcatcttacaacggaacttcgatggcatctccacatgtagctggtgtggcagcgcttgtcaaggcagcgaatccgaacctttcaaacgtgcagcttcgtaatcgcttaaacaacacagcgcaaaacttaggagatgcaaaccactttggaaacggcctagtgaacgcagttgatgccattaactaa

SEQ ID NO: 9 - DNA, 837 bp, artificial sequence
  BspE-clade protease variant
gctcaaacagtaccgtggggagttcctcatgttcaaggtactaaagctcatgcagcggggcatactggaagtggtgtaaaagtagctatactcgatacgggaattgatcgaaatcatgaagatttaaatgtaagaggagggcactctgtattcacacgcagtgcaaaaagagatccttattacgatggtagtggtcatggcacgcacgttgctggaacagtagcggccttaaataatagtgtaggtgtgttaggtgtagcctacaacgcggagctatatgcggtaaaagtattaaataacagtggaagtggtaaatatgcgggaatcgctgaaggaattgaatgggcagtacaaaacaatatgcacattataaatatgagtttaggaggttcgatgagttcttctattttagaagagtggtgtaatattgcctacaattctggtgtgcttgtagtggcggcagctggaaatagtggacgtacgaatggccgtgggaacactgttggttatccagcaaaatatgattctgttatcgcagtagcagcagtttcatctagcaacaatcgtgcaagtttctctagtacaggaaaggcagtggaaattgctgcaccaggtgtaaacattcttagtacgactcctggaaacagctatgcatcttacaacggaacttcgatggcatctccacatgtagctggtgtggcagcgcttgtcttggcagcgaatccgaacctttcaaacgtgcagcttcgtaatcgcttaaacaacacagcgcaaaacttaggagatgcaaaccactttggaaacggcctagtgcgtgcagaagatgccattaactaa

SEQ ID NO: 10 - DNA, 837 bp, artificial sequence
  BspE-clade protease variant
gctcaaacagtaccgtggggagttcctcatgttcaaggtactaaagctcatgcagcggggcatactggaagtggtgtaaaagtagctatactcgatacgggaattgatcgaaatcatgaagatttaaatgtaagaggagggcactctgtattcacagacagtcgtaacagagatccttattacgatggtagtggtcatggcacgcacgttgctggaacagtagcggccttaaataatagtgtaggtgtgttaggtgtagcctacaacgcggagctatatgcggtaaaagtattaaataaccgcggaagtggttcttatgcgggaatcgctgaaggaattgaatgggcagtacaaaaccgtatggacattataaatatgagtttaggaggttcgatgagttcttctattttagaagagtggtgtaatcgcgcctacaattctggtgtgcttgtagtggcggcagctggaaatagtggacgtacgaatggccgtgggaacactgttggttatccagcaaaatatgattctgttatcgcagtagcagcagtttcatctagcaacaatcgtgcaagtttctctagtacaggaaaggcagtggaaattgctgcaccaggtgtaaacattcttagtacgactcctggaaacagctatgcatcttacaacggaacttcgatggcatctccacatgtagctggtgtggcagcgcttgtcaaggcagcgaatccgaacctttcaaacgtgcagcttcgtaatcgcttaaacgatacagcgcaaaacttaggagatgcaaaccactttggaaagggcctagtgcgtgcagaagatgccattaactaa

SEQ ID NO: 11 - DNA, 837 bp, artificial sequence
  BspE-clade protease variant
gctcaaacagtaccgtggggagttcctcatgttcaaggtactgatgctcatgcagcggggcatactggaagtggtgtaaaagtagctatactcgatacgggaattgatcgaaatcatgaagatttaaatgtaagaggagggcgctctgtattcacagacagtcgtaacagagatccttattacgatggtagtggtcatggcacgcacgttgctggaacagtagcggccttaaataatagtgtaggtgtgttaggtgtagcctacaacgcggagctatatgcggtaaaagtattaaataaccgcggaagtggttcttatgcgggaatcgctgaaggaattgaatgggcagtacaaaaccgtatggacattataaatatgagtttaggaggttcgatgcgttcttctattttagaagagtggtgtaatattgcctacaattctggtgtgcttgtagtggcggcagctggaaatagtggacgtacgaatggcaacggggatactgttggttatccagcaaaatatgattctgttatcgcagtagcagcagttgattctagcaacaatcgtgcaagtttctctagtacaggacctgcagtggaaattgctgcaccaggtgtaaacattcttagtacgactcctggaaacagctatgcatcttacaacggaacttcgatggcatctccacatgtagctggtgtggcagcgcttgtcaaggcagcgaatccgaacctttcaaacgtgcagcttcgtaatcgcttaaacaacacagcgcaaaacttaggagatgcaaaccactttggaaagggcctagtgcgtgcagttgatgccattaactaa

SEQ ID NO: 12 - DNA, 837 bp, artificial sequence
  BspE-clade protease variant
gctcaaacagtaccgtggggagttcctcatgttaagggtactaaagctcatgcagcggggcatactggaagtggtgtaaaagtagctatactcgatacgggaattgatgctaatcatgaagatttaaatgtaagaggagggcactctgtattcacagacagtgcaaacagagatccttattacgatggtagtggtcatggcacgcacgttgctggaacagtagcggccttaaataatagtgtaggtgtgttaggtgtagcctacaacgcggagctatatgcggtaaaagtattaaataacagtggaagtggttcttatgcgggaatcgctgaaggaattgaatgggcagtacaaaacaatatgcacattataaatatgagtttaggaggttcgatgagttcttctattttagaagagtggtgtaatattgcctacaattctggtgtgcttgtagtggcggcagctggaaatagtggacgtacgaatggcaacggggatactgttgactatccagcaaaatatgattctgttatcgcagtagcagcagttgattctagcaacaatcgtgcaagtttctctagtacaggacctgcagtggaaattgctgcaccaggtgtaaacattcttagtacgactcctggaaacagctatgcatcttacaacggaacttcgatggcatctccacatgtagctggtgtggcagcgcttgtcttggcagcgaatccgaacctttcaaacgtgcagcttcgtaatcgcttaaacgatacagcgcaaaacttaggagatgcaaaccactttggaaagggcctagtgcgtgcagtttcagccattaactaa

SEQ ID NO: 13 - DNA, 837 bp, artificial sequence
  BspE-clade protease variant
gctcaaacagtaccgtggggagttcctcatgttcaaggtactaaagctcatgcagcggggcatactggaagtggtgtaaaagtagctatactcgatacgggaattgatcgaaatcatgaagatttaaatgtaagaggagggcgctctgtattcacagacagtcgtaacagagatccttattacgatggtagtggtcatggcacgcacgttgctggaacagtagcggccttaaataatagtgtaggtgtgttaggtgtagcctacaacgcggagctatatgcggtaaaagtattaaataaccgcggaagtggttcttatgcgggaatcgctgaaggaattgaatgggcagtacaaaaccgtatggacattataaatatgagtttaggaggttcgatgagttcttctattttagaagagtggtgtaatcgcgcctacaattctggtgtgcttgtagtggcggcagctggaaatagtggacgtacgaatggccgtcgcgatactgttggttatccagcaaaatataactctgttatcgcagtagcagcagttgattctagcaacaatcgtgcaagtttctctagtacaggacctgaagtggaaattgctgcaccaggtgtaaacattcttagtacgactcctggaaacagctatgcatcttacaacggaacttcgatggcatctccacatgtagctggtgtggcagcgcttgtcttggcagcgaatccgcgcctttcaaacgtggagcttcgtaatcgcttaaaagatacagcgcaaaacttaggagatgcaaaccactttggaaacggcctagtgcgtgcagttaaagccattaactaa

SEQ ID NO: 14 - DNA, 837 bp, artificial sequence
  BspE-clade protease variant
gctcaaacagtaccgtggggagttcctcatgttaagggtactgatgctcatgcagcggggcatactggaagtggtcgtaaagtagctatactcgatacgggaattgatgctaatcatgaagatttaaatgtaagaggagggcactctgtattcacagacagtcgtaacagagatccttattacgatggtagtggtcatggcacgcacgttgctggaacagtagcggccttagacaatagtgtaggtgtgttaggtgtagcctacaacgcggagctatatgcggtaaaagtattaaataacagtggaagtggtaaatatgcgggaatcgctgaaggaattgaatgggcagtacaaaacaatatggacattataaatatgagtttaggaggttcgatgagttcttctattttagaagagtggtgtaatcgcgcctacaattctggtgtgcttgtagtggcggcagttggaaatagtggacgtacgaatggccgtggggatactgttggttatccagcaaaatatgattctgttatcgcagtagcagcagtttcatctagcaacaatcgtgcaagtttctctagtacaggacctgaagtggaaattgctgcaccaggtgtaaacattcttagtacgactcctggaaacagctatgcatcttacaacggaacttcgatggcatctccacatgtagctggtgtggcagcgcttgtcttggcagcgaatccgcgcctttcaaacgtggagcttcgtaatcgcttaaacgatacagcgcaacgtttaggagatgcaaaccactttggaaacggcctagtgcgtgcagttaaagccattaactaa

SEQ ID NO: 15 - DNA, 837 bp, artificial sequence
  BspE-clade protease variant
gctcaaacagtaccgtggggagttcctcatgttcaaggtgacgatgctcatgcagcggggcatactggaagtggtgtaaaagtagctatactcgatacgggaattgatcgaaatcatgaagatttaaatgtaagaggagggcactctgtattcacacgcagtgcaaacagagatccttattacgatggtagtggtcatggcacgcacgttgctggaacagtagcggccttaaataatagtgtaggtgtgttaggtgtagcctacaacgcggagctatatgcggtaaaagtattaaataaccgcggaagtggttcttatgcgggaatcgctgaaggaattgaatgggcagtacaaaacaatatggacattataaatatgagtttaggaggttcgatgagttcttctattttagaagagtggtgtaatcgcgcctacaattctggtgtgcttgtagtggcggcagctggaaatagtggacgtacgaatggcaacggggatactgttggttatccagcaaaatattcatctgttatcgcagtagcagcagttgattctagcaacaatcgtgcaagtttctctagtacaggacctgaagtggaaattgctgcaccaggtgtaaacattcttagtacgactcctggaaacagctatgcatcttacaacggaacttcgatggcatctccacatgtagctggtgtggcagcgcttgtcttggcagcgaatccgcgcctttcaaacgtggagcttcgtaatcgcttaaacgatacagcgcaaaacttaggagatgcaaaccactttggaaacggcctagtgcgtgcagttaaagccattaactaa

SEQ ID NO: 16 - DNA, 837 bp, artificial sequence
  BspE-clade protease variant
gctcaaacagtaccgtggggagttcctcatgttcaaggtactaaagctcatgcagcggggcatactggaagtggtgtaaaagtagctatactcgatacgggaattgatcgaaatcatgaagatttaaatgtaagaggagggcactctgtatttacacgcagtgcaaacagagatccttattacgatggtagtggtcatggcacgcacgttgctggaacagtagcggccttaaataatagtgtaggtgtgttaggtgtagcctacaacgcggagctatatgcggtaaaagtattaaataaccgcggaagtggttcttatgcgggaatcgctgaaggaattgaatgggcagtacaaaaccgtatggacattataaatatgagtttaggaggttcgatgagttcttctattttagaagagtggtgtaatcgcgcctacaattctggtgtgcttgtagtggcggcagctggaaatagtggacgtacgaatggccgtcgcgatactgttggttatccagcaaaatattcatctgttatcgcagtagcagcagttgattctagcaacaatcgtgcaagtttctctagtacaggacctgcagtggaaattgctgcaccaggtgtaaacattcttagtacgactcctggaaacagctatgcatcttacaacggaacttcgatggcatctccacatgtagctggtgtggcagcgcttgtcttggcagcgaatccgcgcctttcaaacgtggagcttcgtaatcgcttaaacaacacagcgcaaaacttaggagatgcaaaacactttggaaacggcctagtgcgtgcagttaaagccattaactaa

SEQ ID NO: 17 - DNA, 837 bp, artificial sequence
  BspE-clade protease variant
gctcaaacagtaccgtggggagttcctcatgttaagggtactgatgctcatgcagcggggcatactggaagtggtcgtaaagtagctatactcgatacgggaattgatgctaatcatgaagatttaaatgtaagaggagggcgctctgtattcacagacagtcgtaacagagatccttattacgatggtagtggtcatggcacgcacgttgctggaacagtagcggccttagacaatagtgtaggtgtgttaggtgtagcctacaacgcggagctatatgcggtaaaagtattaaataaccgcggaagtggttcttatgcgggaatcgctgaaggaattgaatgggcagtacaaaacaatatgcacattataaatatgagtttaggaggttcgatgagttcttctattttagaagagtggtgtaatcgcgcctacaattctggtgtgcttgtagtggcggcagctggaaatagtggacgtacgaatggccgtgggaacactgttggttatccagcaaaatatccttctgttatcgcagtagcagcagtttcatctagcaacaatcgtgcaagtttctctagtacaggacctgcagtggaaattgctgcaccaggtgtaaacattcttagtacgactcctggaaacagctatgcatctcgcaacggaacttcgatggcatctccacatgtagctggtgtggcagcgcttgtcttggcagcgaatccgcgcctttcaaacgtggagcttcgtaatcgcttaaacaacacagcgcaaaacttaggagatgcaaaccactttggaaacggcctagtgaacgcagttgatgccattaactaa

SEQ ID NO: 18 - protein, 278 aa, artificial sequence
  BspE-clade protease variant
AQTVPWGVPHVQGTDAHAAGHTGSGVKVAILDTGIDANHEDLNVRGGHSVFTGSANRDPYYDGSGHGTHVAGTVAALNNSVGVLGVAYNAELYAVKVLNNRGSGSYAGIAEGIEWAVQNRMDIINMSLGGSMSSSILEEWCNRAYNSGVLVVAAAGNSGRTNGRGNTVGYPAKYDSVIAVAAVSSSNNRASFSSTGKAVEIAAPGVNILSTTPGNSYASYNGTSMASPHVAGVAALVKAANPNLSNVQLRNRLNNTAQNLGDANHFGNGLVNAVDAIN

SEQ ID NO: 19 - protein, 278 aa, artificial sequence
  BspE-clade protease variant
AQTVPWGVPHVQGTKAHAAGHTGSGVKVAILDTGIDRNHEDLNVRGGHSVFTRSAKRDPYYDGSGHGTHVAGTVAALNNSVGVLGVAYNAELYAVKVLNNSGSGKYAGIAEGIEWAVQNNMHIINMSLGGSMSSSILEEWCNIAYNSGVLVVAAAGNSGRTNGRGNTVGYPAKYDSVIAVAAVSSSNNRASFSSTGKAVEIAAPGVNILSTTPGNSYASYNGTSMASPHVAGVAALVLAANPNLSNVQLRNRLNNTAQNLGDANHFGNGLVRAEDAIN

SEQ ID NO: 20 - protein, 278 aa, artificial sequence
  BspE-clade protease variant
AQTVPWGVPHVQGTKAHAAGHTGSGVKVAILDTGIDRNHEDLNVRGGHSVFTDSRNRDPYYDGSGHGTHVAGTVAALNNSVGVLGVAYNAELYAVKVLNNRGSGSYAGIAEGIEWAVQNRMDIINMSLGGSMSSSILEEWCNRAYNSGVLVVAAAGNSGRTNGRGNTVGYPAKYDSVIAVAAVSSSNNRASFSSTGKAVEIAAPGVNILSTTPGNSYASYNGTSMASPHVAGVAALVKAANPNLSNVQLRNRLNDTAQNLGDANHFGKGLVRAEDAIN

SEQ ID NO: 21 - protein, 278 aa, artificial sequence
  BspE-clade protease variant
AQTVPWGVPHVQGTDAHAAGHTGSGVKVAILDTGIDRNHEDLNVRGGRSVFTDSRNRDPYYDGSGHGTHVAGTVAALNNSVGVLGVAYNAELYAVKVLNNRGSGSYAGIAEGIEWAVQNRMDIINMSLGGSMRSSILEEWCNIAYNSGVLVVAAAGNSGRTNGNGDTVGYPAKYDSVIAVAAVDSSNNRASFSSTGPAVEIAAPGVNILSTTPGNSYASYNGTSMASPHVAGVAALVKAANPNLSNVQLRNRLNNTAQNLGDANHFGKGLVRAVDAIN

SEQ ID NO: 22 - protein, 278 aa, artificial sequence
  BspE-clade protease variant
AQTVPWGVPHVKGTKAHAAGHTGSGVKVAILDTGIDANHEDLNVRGGHSVFTDSANRDPYYDGSGHGTHVAGTVAALNNSVGVLGVAYNAELYAVKVLNNSGSGSYAGIAEGIEWAVQNNMHIINMSLGGSMSSSILEEWCNIAYNSGVLVVAAAGNSGRTNGNGDTVDYPAKYDSVIAVAAVDSSNNRASFSSTGPAVEIAAPGVNILSTTPGNSYASYNGTSMASPHVAGVAALVLAANPNLSNVQLRNRLNDTAQNLGDANHFGKGLVRAVSAIN

SEQ ID NO: 23 - protein, 278 aa, artificial sequence
  BspE-clade protease variant
AQTVPWGVPHVQGTKAHAAGHTGSGVKVAILDTGIDRNHEDLNVRGGRSVFTDSRNRDPYYDGSGHGTHVAGTVAALNNSVGVLGVAYNAELYAVKVLNNRGSGSYAGIAEGIEWAVQNRMDIINMSLGGSMSSSILEEWCNRAYNSGVLVVAAAGNSGRTNGRRDTVGYPAKYNSVIAVAAVDSSNNRASFSSTGPEVEIAAPGVNILSTTPGNSYASYNGTSMASPHVAGVAALVLAANPRLSNVELRNRLKDTAQNLGDANHFGNGLVRAVKAIN

SEQ ID NO: 24 - protein, 278 aa, artificial sequence
  BspE-clade protease variant
AQTVPWGVPHVKGTDAHAAGHTGSGRKVAILDTGIDANHEDLNVRGGHSVFTDSRNRDPYYDGSGHGTHVAGTVAALDNSVGVLGVAYNAELYAVKVLNNSGSGKYAGIAEGIEWAVQNNMDIINMSLGGSMSSSILEEWCNRAYNSGVLVVAAVGNSGRTNGRGDTVGYPAKYDSVIAVAAVSSSNNRASFSSTGPEVEIAAPGVNILSTTPGNSYASYNGTSMASPHVAGVAALVLAANPRLSNVELRNRLNDTAQRLGDANHFGNGLVRAVKAIN

SEQ ID NO: 25 - protein, 278 aa, artificial sequence
  BspE-clade protease variant
AQTVPWGVPHVQGDDAHAAGHTGSGVKVAILDTGIDRNHEDLNVRGGHSVFTRSANRDPYYDGSGHGTHVAGTVAALNNSVGVLGVAYNAELYAVKVLNNRGSGSYAGIAEGIEWAVQNNMDIINMSLGGSMSSSILEEWCNRAYNSGVLVVAAAGNSGRTNGNGDTVGYPAKYSSVIAVAAVDSSNNRASFSSTGPEVEIAAPGVNILSTTPGNSYASYNGTSMASPHVAGVAALVLAANPRLSNVELRNRLNDTAQNLGDANHFGNGLVRAVKAIN

SEQ ID NO: 26 - protein, 278 aa, artificial sequence
  BspE-clade protease variant
AQTVPWGVPHVQGTKAHAAGHTGSGVKVAILDTGIDRNHEDLNVRGGHSVFTRSANRDPYYDGSGHGTHVAGTVAALNNSVGVLGVAYNAELYAVKVLNNRGSGSYAGIAEGIEWAVQNRMDIINMSLGGSMSSSILEEWCNRAYNSGVLVVAAAGNSGRTNGRRDTVGYPAKYSSVIAVAAVDSSNNRASFSSTGPAVEIAAPGVNILSTTPGNSYASYNGTSMASPHVAGVAALVLAANPRLSNVELRNRLNNTAQNLGDAKHFGNGLVRAVKAIN

SEQ ID NO: 27 - protein, 278 aa, artificial sequence
  BspE-clade protease variant
AQTVPWGVPHVKGTDAHAAGHTGSGRKVAILDTGIDANHEDLNVRGGRSVFTDSRNRDPYYDGSGHGTHVAGTVAALDNSVGVLGVAYNAELYAVKVLNNRGSGSYAGIAEGIEWAVQNNMHIINMSLGGSMSSSILEEWCNRAYNSGVLVVAAAGNSGRTNGRGNTVGYPAKYPSVIAVAAVSSSNNRASFSSTGPAVEIAAPGVNILSTTPGNSYASRNGTSMASPHVAGVAALVLAANPRLSNVELRNRLNNTAQNLGDANHFGNGLVNAVDAIN

SEQ ID NO: 28 - protein, 307 aa, Bacillus sp.
  misc_feature (1)..(307): Bacillus sp. SWT183
AQTVPWGVPHVQGTDAHAAGHTGSGVKVAILDTGIDRNHEDLNVRGGHSVFTDSANSDPYYDGSGHGTHVAGTVAALNNSVGVLGVAYNAELYAVKVLNNSGSGSYAGIAQGIEWAVQNNMDIINMSLGGSMSSSILEEWCNIAYNSGVLVVAAAGNSGRTNGRGDTVGYPAKYDSVIAVAAVDSSNNRASFSSTGSAVEIAAPGVNILSTTPGNSYASYNGTSMASPHVAGVAALVWAANPNLSNVELRNRLNDTAQNLGDANHFGHGLVRAVDAINGTSSGDNGGGDDGGSGPTKPGNGKGNGKN

SEQ ID NO: 29 - protein, 307 aa, Bacillus sp.
  MISC_FEATURE (1)..(307): Bacillus sp. KSM-LD1
AQTVPWGVPHVQGTDAHAAGHTGSGVKVAILDTGIDRNHEDLNVRGGHSVFTDSANRDPYYDGSGHGTHVAGTVAALNNSVGVLGVAYNAELYAVKVLNNSGSGSYAGIAEGIEWAVNNGMDIINMSLGGSMSSSILEEWCNIAYNSGVLVVAAAGNSGRTNGRGDTVGYPAKYDSVIAVAAVDSSNNRASFSSTGPAVEIAAPGVNILSTTPGNSYASYNGTSMASPHVAGVAALVLAANPNLSNVELRNRLNDTAQNLGDANHFGNGLVRAVDAINGTSSGDNGGGDDGGSEPTKPGNGKGNGRN

SEQ ID NO: 30 - protein, 275 aa, Bacillus amyloliquefaciens [sequence omitted]

SEQ ID NO: 31 - protein, 269 aa, Bacillus lentus
AQSVPWGISRVQAPAAHNRGLTGSGVKVAVLDTGISTHPDLNIRGGASFVPGEPSTQDGNGHGTHVAGTIAALNNSIGVLGVAPSAELYAVKVLGASGSGSVSSIAQGLEWAGNNGMHVANLSLGSPSPSATLEQAVNSATSRGVLVVAASGNSGAGSISYPARYANAMAVGATDQNNNRASFSQYGAGLDIVAPGVNVQSTYPGSTYASLNGTSMATPHVAGAAALVKQKNPSWSNVQIRNHLKNTATSLGSTNLYGSGLVNAEAATR

SEQ ID NO: 32 - protein, 275 aa, Bacillus sp.
  misc_feature (1)..(275): Bacillus sp. SprC
AQTVPWGIPHIKADKAHAAGVTGSGVKVAILDTGIDANHADLNVKGGASFVSGEPNALQDGNGHGTHVAGTVAALNNTTGVLGVAYNADLYAVKVLSASGSGTLSGIAQGIEWSISNGMNVINMSLGGSSGSTALQQACNNAYNRGIVVIAAAGNSGSSGNRNTMGYPARYSSVIAVGAVSSNNTRASFSSVGSELEVMAPGVNILSTTPGNNYASFNGTSMAAPHVAGAAALIKAKYPSMTNVQIRERLKNTATNLGDPFFYGKGVINVESALQ

SEQ ID NO: 33 - protein, 274 aa, Bacillus licheniformis
AQTVPYGIPLIKADKVQAQGFKGANVKVAVLDTGIQASHPDLNVVGGASFVAGEAYNTDGNGHGTHVAGTVAALDNTTGVLGVAPSVSLYAVKVLNSSGSGSYSGIVSGIEWATTNGMDVINMSLGGASGSTAMKQAVDNAYARGVVVVAAAGNSGSSGNTNTIGYPAKYDSVIAVGAVDSNSNRASFSSVGAELEVMAPGAGVYSTYPTNTYATLNGTSMASPHVAGAAALILSKHPNLSASQVRNRLSSTATYLGSSFYYGKGLINVEAAAQ

SEQ ID NO: 34 - protein, 280 aa, Bacillus sp.
  misc_feature (1)..(280): Bacillus sp. GX6638 (ATCC 53278)
AQTVPWGVPHVQGTDAHAAGHTGSGVKVAILDTGIDRNHEDLNVRGGHSVFTDSANRDPYYDGSGHGTHVAGTVAALNNSVGVLGVAYNAELYAVKVLNNSGSGSYAGIAEGIEWAVQNNMDIINMSLGGSMSSSILEEWCNIAYNSGVLVVAAAGNSGRTNGRGDTVGYPAKYDSVIAVAAVDSSNNRASFSSTGPAVEIAAPGVNILSTTPGNSYASYNGTSMASPHVAGVAALVLAANPNLSNVELRNRLNDTAQNLGDANHFGNGLVRAVDAINGT

SEQ ID NO: 35 - protein, 35 aa, artificial sequence
  Motif
  MISC_FEATURE (1)..(35): X is any amino acid
DTGIXXXHXDLXXXGGXSVFXXXXXXXXXXDXXGH

SEQ ID NO: 36 - protein, 35 aa, artificial sequence
  Motif
  MISC_FEATURE (1)..(35): X is any amino acid
DTGIXXXHXDLXXXGGXSVFXXXXXXDPXXDXXGH

SEQ ID NO: 37 - protein, 35 aa, artificial sequence
  Motif
  MISC_FEATURE (1)..(35): X is any amino acid
DTGIXXXHXDLNVXGGXSVFXXXXXXXXXXDXXGH

SEQ ID NO: 38 - protein, 35 aa, artificial sequence
  Motif
  MISC_FEATURE (1)..(35): X is any amino acid
DTGIXXXHXDLNVXGGXSVFXXXXXXDPXXDXXGH

SEQ ID NO: 39 - protein, 35 aa, artificial sequence
  Motif
  MISC_FEATURE (1)..(35): X is any amino acid
DTGIDXXHXDLNVXGGXSVFXXXXXXXXXXDXXGH

SEQ ID NO: 40 - protein, 35 aa, artificial sequence
  Motif
  MISC_FEATURE (1)..(35): X is any amino acid
DTGIDXNHXDLNVRGGXSVFTXXXXXDPXXDXXGH

SEQ ID NO: 41 - protein, 35 aa, artificial sequence
  Motif
  MISC_FEATURE (1)..(35): X is any amino acid
DTGIDXNHXDLNVRGGXSVFTXXXXXDPYYDXXGH